European Patent Specification EP 3 648 789 B9, published September 27, 2023. Title: Compositions and methods for the treatment of myopathies. Applicant: Université de Strasbourg et al. The sequence listing filed with the application follows.

SEQUENCE LISTING (29 sequences)

SEQ ID NO: 1 - protein, 571 aa, Homo sapiens
MEEPPLLPGENIKDMAKDVTYICPFTGAVRGTLTVTNYRLYFKSMERDPPFVLDASLGVINRVEKIGGASSRGENSYGLETVCKDIRNLRFAHKPEGRTRRSIFENLMKYAFPVSNNLPLFAFEYKEVFPENGWKLYDPLLEYRRQGIPNESWRITKINERYELCDTYPALLVVPANIPDEELKRVASFRSRGRIPVLSWIHPESQATITRCSQPMVGVSGKRSKEDEKYLQAIMDSNAQSHKIFIFDARPSVNAVANKAKGGGYESEDAYQNAELVFLDIHNIHVMRESLRKLKEIVYPNIEETHWLSNLESTHWLEHIKLILAGALRIADKVESGKTSVVVHCSDGWDRTAQLTSLAMLMLDGYYRTIRGFEVLVEKEWLSFGHRFQLRVGHGDKNHADADRSPVFLQFIDCVWQMTRQFPTAFEFNEYFLITILDHLYSCLFGTFLCNSEQQRGKENLPKRTVSLWSYINSQLEDFTNPLYGSYSNHVLYPVASMRHLELWVGYYIRWNPRMKPQEPIHNRYKELLAKRAELQKKVEELQREISNRSTSSSERASSPAQCVTPVQTVV

SEQ ID NO: 2 - DNA, 1716 bp, Homo sapiens
atggaagaaccacccttgcttccaggagaaaatattaaagacatggccaaagatgtaacttatatatgtccattcactggcgctgtacgaggaactctgactgtcacgaattataggttatatttcaaaagcatggaacgggatcccccatttgttttagatgcttcccttggtgtgataaatagagtagaaaaaattggtggtgcttctagtcgaggtgaaaattcttatggactagaaactgtgtgtaaggatattaggaatttacgatttgctcataaacctgaggggcggacaagaagatccatatttgagaatctaatgaaatatgcatttcctgtctctaataacctgcctctttttgcttttgaatacaaagaagtattccctgaaaatgggtggaagctatatgaccctcttttagagtatagaaggcagggaattccaaatgaaagctggagaataacaaagataaatgaacgatatgaactttgtgatacataccctgccctcctggttgtgccagcaaatattcctgatgaagaattaaagagagtggcatccttcagatcaagaggccgtatcccagttttatcatggattcatcctgaaagtcaagccacaatcactcggtgtagccagcccatggttggagtgagtggaaagcgaagcaaagaagatgaaaaataccttcaagctatcatggattccaatgcccagtctcacaaaatctttatatttgatgcccggccaagtgttaatgctgttgccaacaaggcaaagggtggaggttatgaaagtgaagatgcctatcaaaatgctgaactagttttcctggatatccacaatattcatgttatgagagaatcattacgaaaacttaaggagattgtgtaccccaacattgaggaaacccactggttgtctaacttggaatctactcattggctagaacatattaagcttattcttgcaggggctcttaggattgctgacaaggtagagtcagggaagacgtctgtggtagtgcattgcagtgatggttgggatcgcacagctcagctcacttcccttgccatgctcatgttggatggatactatcgaaccatccgaggatttgaagtccttgtggagaaagaatggctaagttttggacatcgatttcaactaagagttggccatggagataagaaccatgcagatgcagacagatcgcctgtttttcttcaatttattgactgtgtctggcagatgacaagacagtttcctaccgcatttgaattcaatgagtattttctcattaccattttggaccacctatacagctgcttattcggaacattcctctgtaatagtgaacaacagagaggaaaagagaatcttcctaaaaggactgtgtcactgtggtcttacataaacagccagctggaagacttcactaatcctctctatgggagctattccaatcatgtcctttatccagtagccagcatgcgccacctagagctctgggtgggatattacataaggtggaatccacggatgaaaccacaggaacctattcacaacagatacaaagaacttcttgctaaacgagcagagcttcagaaaaaagtagaggaactacagagagagatttctaaccgatcaacctcatcctcagagagagccagctctcctgcacagtgtgtcactcctgtccaaactgttgtataa

SEQ ID NO: 3 - DNA, 4789 bp, Homo sapiens
agatgtcgcgcggccggacacagccagcacggagagtcgatgccggcgtctgagctgcgcagtggggtcttcccgctgcccagcagcctacaggcgcggtgcactctgggggaacatggccgcttccggtctccctcccgggccggcgctggcctgactgcggccccggtccgtagcactccgccctccgcttctcccgccctgtagccgcgaagactgcttcagcctttccctgtgctgcccctgccgcgcgatggagaagagctcgagctgcgagagtcttggctcccagccggcggcggctcggccgcccagcgtggactccttgtccagttaatgtgttaagagccattgacatttgaagatcatcagaagtgaagataaaacatctcaaaaattataattgcctccacttctcattcagagaattcagtgcatacaaaatcagcttctgttgtatcatcagattccatttcaacttctgccgacaacttttctcctgatttgaggagggagtctcgctctatcccctaggctggagtgcattggcgccatctcggctcatttgcaacctctgtctcccgggttcaagcgattctcctgcctcagcttcccgaggagctgggattacaggtcctgagggagtctaacaagttagcagaaatggaagaaccacccttgcttccaggagaaaatattaaagacatggccaaagatgtaacttatatatgtccattcactggcgctgtacgaggaactctgactgtcacgaattataggttatatttcaaaagcatggaacgggatcccccatttgttttagatgcttcccttggtgtgataaatagagtagaaaaaattggtggtgcttctagtcgaggtgaaaattcttatggactagaaactgtgtgtaaggatattaggaatttacgatttgctcataaacctgaggggcggacaagaagatccatatttgagaatctaatgaaatatgcatttcctgtctctaataacctgcctctttttgcttttgaatacaaagaagtattccctgaaaatgggtggaagctatatgaccctcttttagagtatagaaggcagggaattccaaatgaaagctggagaataacaaagataaatgaacgatatgaactttgtgatacataccctgccctcctggttgtgccagcaaatattcctgatgaagaattaaagagagtggcatccttcagatcaagaggccgtatcccagttttatcatggattcatcctgaaagtcaagccacaatcactcggtgtagccagcccatggttggagtgagtggaaagcgaagcaaagaagatgaaaaataccttcaagctatcatggattccaatgcccagtctcacaaaatctttatatttgatgcccggccaagtgttaatgctgttgccaacaaggcaaagggtggaggttatgaaagtgaagatgcctatcaaaatgctgaactagttttcctggatatccacaatattcatgttatgagagaatcattacgaaaacttaaggagattgtgtaccccaacattgaggaaacccactggttgtctaacttggaatctactcattggctagaacatattaagcttattcttgcaggggctcttaggattgctgacaaggtagagtcagggaagacgtctgtggtagtgcattgcagtgatggttgggatcgcacagctcagctcacttcccttgccatgctcatgttggatggatactatcgaaccatccgaggatttgaagtccttgtggagaaagaatggctaagttttggacatcgatttcaactaagagttggccatggagataagaaccatgcagatgcagacagatcgcctgtttttcttcaatttattgactgtgtctggcagatgacaagacagtttcctaccgcatttgaattcaatgagtattttctcattaccattttggaccacctatacagctgcttattcggaacattcctctgtaatagtgaacaacagagaggaaaagagaatcttcctaaaaggactgtgtcactgtggtcttacataaacagccagctggaagacttcactaatcctctctatgggagctattccaatcatgtcctttatccagtagccagcatgcgccacctagagctctgggtgggatattacataaggtggaatccacggatgaaaccacaggaacctattcacaacagatacaaagaacttcttgctaaacgagcagagcttcagaaaaaagtagaggaactacagagagagatttctaaccgatcaacctcatcctcagagagagccagctctcctgcacagtgtgtcactcctgtccaaactgttgtataaaggactgtaagatcaggggcatcattgctatacactcttgattacactggcagctctatgagtagaaagtcttcggaatttagaacccatctatgagagaaagttcagtcactttatttattttaaatctctctaggatgagtttagaactgtagcagtgcaggtggcttaagtgaagtaactccatatgtaattacatgattatgatactaatcttttaagtatccaaagaatattaaaatacttcaatcctggattcacagtgggaacaagtttctattaaaaggcaaatgctgttacaaatttttggcatctggtaatattaaaaccattttagaaatacactctgtgctcactgtgcagaggaacatcagttttcaaaccaacactgaaattctgtggcatcacatatattgggccttgatgtcatgacagatcaaaatcatttgatatccctttctccattctaggtttttctttttttcagtaactgatttaccttgatcacttttcaacttccatattcttcatatagtaaaaggcaaagtgttgaagatactacggtgtggtagtagttgaaaattattgccgtcattatttacatacttaagacatattagcaagttgatccaaaatgggaggccttatagatgtgcttgggggaaaatgaaggggagaaagtagccatacaggagttcaaagaattccatgcccttcagattagcccaattaccagaaacatcatgaaagatattttaaaaactaattatttactacagtgtatttcacttgtcttgtgtgtctgaacacacagaagctaattagcaagtttttaagaagtatttaaaaatcttactaggattgacattttttctgaattctgtataaatagcttatagtgagaagtactgtgctcaaattttacatttttttcctttgcaaattctgtaatttcactcaacgattaagtctaccaaagaacacactgcatgtaaaagatgtattacaatctcaaagccagtaaaagaaatcttgcttcactgttcacctgctacaagtaagagtttggtgctggtagaaacatttgactctgatgtctattttattctacataagagccatatgtaatgtactgtaacaaaggagcttcttgtccccttggtcttttaattaaaagaaattccaactgacttttaaactttgttcttgtccaaagttgccatttcttttttttccccagaaatatttggaaattattggaggaatatgcaccccagatgaaaatgttcagtttgtacccatttttccttaaccaacacccaaatcaaacaattaaaatatacagtgtttttccactcactaattcactatacagagagtctgaaccttagcctccctcttggtcttgcagtgaggaagtttctattagtatatccaatttagcaaaattggtaccaaaatgatttctttggtaattgtgtgaaatataagctttttaacagggcatttaagtggctagcaaatcagtaattaaaaattaagctttctactccaagtatttcacaaacgcatctgccattttcctcatttaaaccttggttatcttggcctgataccacataaaagaatgtagaatggctgaagagatcaagaatttaaagcttctagtcttaacatacttgcatccacttcaaattcaaatcaaaagccagggaaatctaagtgcaaccctaccacttctctgctgagaaccttccagtggttcccctcaccttctgcagaagtctccaatatggagtacatgcacttgggcatttaatatataccactggtgtgtgtgggagggagggaggaggaatactagccctttttatatatttacacaagcaaaacttttaaatatttgaattgacagttacatgtttcataactttgtatgtctattggttgtgcaggtgtaattttttccctttttgattagggttacaaaatttagagaccagtatgattaagttgaagctccttagcctccttcgacctagtctctgcatacctcaacttttacgtaccaatgctactctgctgttcacaattgcctcatgtaatctgcagattcctgcctccccactttggttcagtctgtcttgtgcacctggaacaactgttctcccttgtgactaattcctattttctagagtttaggcatcatctcttcctttgggaagttatctgattcacgactgccttctctgacatccccaccttcctctgtgcccccatagcactgtgtataccgctactaccactgcaattcacattatattggaatgaacaattcacatgtctaccacaagtctgtaaacataaccttatttgaaatgaattgcaataaagctctgttacaacgtaa

SEQ ID NO: 4 - DNA, 4666 bp, Homo sapiens
agatgtcgcgcggccggacacagccagcacggagagtcgatgccggcgtctgagctgcgcagtggggtcttcccgctgcccagcagcctacaggcgcggtgcactctgggggaacatggccgcttccggtctccctcccgggccggcgctggcctgactgcggccccggtccgtagcactccgccctccgcttctcccgccctgtagccgcgaagactgcttcagcctttccctgtgctgcccctgccgcgcgatggagaagagctcgagctgcgagagtcttggctcccagccggcggcggctcggccgcccagcgtggactccttgtccagttaatgtgttaagagccattgacatttgaagatcatcagaagtgaagataaaacatctcaaaaattataattgcctccacttctcattcagagaattcagtgcatacaaaatcagcttctgttgtatcatcagattccatttcaacttctgccgacaacttttctcctgatttgagggtcctgagggagtctaacaagttagcagaaatggaagaaccacccttgcttccaggagaaaatattaaagacatggccaaagatgtaacttatatatgtccattcactggcgctgtacgaggaactctgactgtcacgaattataggttatatttcaaaagcatggaacgggatcccccatttgttttagatgcttcccttggtgtgataaatagagtagaaaaaattggtggtgcttctagtcgaggtgaaaattcttatggactagaaactgtgtgtaaggatattaggaatttacgatttgctcataaacctgaggggcggacaagaagatccatatttgagaatctaatgaaatatgcatttcctgtctctaataacctgcctctttttgcttttgaatacaaagaagtattccctgaaaatgggtggaagctatatgaccctcttttagagtatagaaggcagggaattccaaatgaaagctggagaataacaaagataaatgaacgatatgaactttgtgatacataccctgccctcctggttgtgccagcaaatattcctgatgaagaattaaagagagtggcatccttcagatcaagaggccgtatcccagttttatcatggattcatcctgaaagtcaagccacaatcactcggtgtagccagcccatggttggagtgagtggaaagcgaagcaaagaagatgaaaaataccttcaagctatcatggattccaatgcccagtctcacaaaatctttatatttgatgcccggccaagtgttaatgctgttgccaacaaggcaaagggtggaggttatgaaagtgaagatgcctatcaaaatgctgaactagttttcctggatatccacaatattcatgttatgagagaatcattacgaaaacttaaggagattgtgtaccccaacattgaggaaacccactggttgtctaacttggaatctactcattggctagaacatattaagcttattcttgcaggggctcttaggattgctgacaaggtagagtcagggaagacgtctgtggtagtgcattgcagtgatggttgggatcgcacagctcagctcacttcccttgccatgctcatgttggatggatactatcgaaccatccgaggatttgaagtccttgtggagaaagaatggctaagttttggacatcgatttcaactaagagttggccatggagataagaaccatgcagatgcagacagatcgcctgtttttcttcaatttattgactgtgtctggcagatgacaagacagtttcctaccgcatttgaattcaatgagtattttctcattaccattttggaccacctatacagctgcttattcggaacattcctctgtaatagtgaacaacagagaggaaaagagaatcttcctaaaaggactgtgtcactgtggtcttacataaacagccagctggaagacttcactaatcctctctatgggagctattccaatcatgtcctttatccagtagccagcatgcgccacctagagctctgggtgggatattacataaggtggaatccacggatgaaaccacaggaacctattcacaacagatacaaagaacttcttgctaaacgagcagagcttcagaaaaaagtagaggaactacagagagagatttctaaccgatcaacctcatcctcagagagagccagctctcctgcacagtgtgtcactcctgtccaaactgttgtataaaggactgtaagatcaggggcatcattgctatacactcttgattacactggcagctctatgagtagaaagtcttcggaatttagaacccatctatgagagaaagttcagtcactttatttattttaaatctctctaggatgagtttagaactgtagcagtgcaggtggcttaagtgaagtaactccatatgtaattacatgattatgatactaatcttttaagtatccaaagaatattaaaatacttcaatcctggattcacagtgggaacaagtttctattaaaaggcaaatgctgttacaaatttttggcatctggtaatattaaaaccattttagaaatacactctgtgctcactgtgcagaggaacatcagttttcaaaccaacactgaaattctgtggcatcacatatattgggccttgatgtcatgacagatcaaaatcatttgatatccctttctccattctaggtttttctttttttcagtaactgatttaccttgatcacttttcaacttccatattcttcatatagtaaaaggcaaagtgttgaagatactacggtgtggtagtagttgaaaattattgccgtcattatttacatacttaagacatattagcaagttgatccaaaatgggaggccttatagatgtgcttgggggaaaatgaaggggagaaagtagccatacaggagttcaaagaattccatgcccttcagattagcccaattaccagaaacatcatgaaagatattttaaaaactaattatttactacagtgtatttcacttgtcttgtgtgtctgaacacacagaagctaattagcaagtttttaagaagtatttaaaaatcttactaggattgacattttttctgaattctgtataaatagcttatagtgagaagtactgtgctcaaattttacatttttttcctttgcaaattctgtaatttcactcaacgattaagtctaccaaagaacacactgcatgtaaaagatgtattacaatctcaaagccagtaaaagaaatcttgcttcactgttcacctgctacaagtaagagtttggtgctggtagaaacatttgactctgatgtctattttattctacataagagccatatgtaatgtactgtaacaaaggagcttcttgtccccttggtcttttaattaaaagaaattccaactgacttttaaactttgttcttgtccaaagttgccatttcttttttttccccagaaatatttggaaattattggaggaatatgcaccccagatgaaaatgttcagtttgtacccatttttccttaaccaacacccaaatcaaacaattaaaatatacagtgtttttccactcactaattcactatacagagagtctgaaccttagcctccctcttggtcttgcagtgaggaagtttctattagtatatccaatttagcaaaattggtaccaaaatgatttctttggtaattgtgtgaaatataagctttttaacagggcatttaagtggctagcaaatcagtaattaaaaattaagctttctactccaagtatttcacaaacgcatctgccattttcctcatttaaaccttggttatcttggcctgataccacataaaagaatgtagaatggctgaagagatcaagaatttaaagcttctagtcttaacatacttgcatccacttcaaattcaaatcaaaagccagggaaatctaagtgcaaccctaccacttctctgctgagaaccttccagtggttcccctcaccttctgcagaagtctccaatatggagtacatgcacttgggcatttaatatataccactggtgtgtgtgggagggagggaggaggaatactagccctttttatatatttacacaagcaaaacttttaaatatttgaattgacagttacatgtttcataactttgtatgtctattggttgtgcaggtgtaattttttccctttttgattagggttacaaaatttagagaccagtatgattaagttgaagctccttagcctccttcgacctagtctctgcatacctcaacttttacgtaccaatgctactctgctgttcacaattgcctcatgtaatctgcagattcctgcctccccactttggttcagtctgtcttgtgcacctggaacaactgttctcccttgtgactaattcctattttctagagtttaggcatcatctcttcctttgggaagttatctgattcacgactgccttctctgacatccccaccttcctctgtgcccccatagcactgtgtataccgctactaccactgcaattcacattatattggaatgaacaattcacatgtctaccacaagtctgtaaacataaccttatttgaaatgaattgcaataaagctctgttacaacgtaa

SEQ ID NO: 5 - DNA, 4862 bp, Homo sapiens
agatgtcgcgcggccggacacagccagcacggagagtcgatgccggcgtctgagctgcgcagtggggtcttcccgctgcccagcagcctacaggcgcggtgcactctgggggaacatggccgcttccggtctccctcccgggccggcgctggcctgactgcggccccggtccgtagcactccgccctccgcttctcccgccctgtagccgcgaagactgcttcagcctttccctgtgctgcccctgccgcgcgatggagaagagctcgagctgcgagagtcttggctcccagccggcggcggctcggccgcccagcgtggactccttgtccagttaatgtgttaagagccattgacatttgaagatcatcagaagtgaagataaaacatctcaaaaattataattgcctccacttctcattcagagaattcagtgcatacaaaatcagcttctgttgtatcatcagattccatttcaacttctgccgacaacttttctcctgatttgaggcccatgcagtccagttcgggagctaagtcacttaaacactgtgtgatagttcctacacatctcattatagtttagggagtctcgctctatcccctaggctggagtgcattggcgccatctcggctcatttgcaacctctgtctcccgggttcaagcgattctcctgcctcagcttcccgaggagctgggattacaggtcctgagggagtctaacaagttagcagaaatggaagaaccacccttgcttccaggagaaaatattaaagacatggccaaagatgtaacttatatatgtccattcactggcgctgtacgaggaactctgactgtcacgaattataggttatatttcaaaagcatggaacgggatcccccatttgttttagatgcttcccttggtgtgataaatagagtagaaaaaattggtggtgcttctagtcgaggtgaaaattcttatggactagaaactgtgtgtaaggatattaggaatttacgatttgctcataaacctgaggggcggacaagaagatccatatttgagaatctaatgaaatatgcatttcctgtctctaataacctgcctctttttgcttttgaatacaaagaagtattccctgaaaatgggtggaagctatatgaccctcttttagagtatagaaggcagggaattccaaatgaaagctggagaataacaaagataaatgaacgatatgaactttgtgatacataccctgccctcctggttgtgccagcaaatattcctgatgaagaattaaagagagtggcatccttcagatcaagaggccgtatcccagttttatcatggattcatcctgaaagtcaagccacaatcactcggtgtagccagcccatggttggagtgagtggaaagcgaagcaaagaagatgaaaaataccttcaagctatcatggattccaatgcccagtctcacaaaatctttatatttgatgcccggccaagtgttaatgctgttgccaacaaggcaaagggtggaggttatgaaagtgaagatgcctatcaaaatgctgaactagttttcctggatatccacaatattcatgttatgagagaatcattacgaaaacttaaggagattgtgtaccccaacattgaggaaacccactggttgtctaacttggaatctactcattggctagaacatattaagcttattcttgcaggggctcttaggattgctgacaaggtagagtcagggaagacgtctgtggtagtgcattgcagtgatggttgggatcgcacagctcagctcacttcccttgccatgctcatgttggatggatactatcgaaccatccgaggatttgaagtccttgtggagaaagaatggctaagttttggacatcgatttcaactaagagttggccatggagataagaaccatgcagatgcagacagatcgcctgtttttcttcaatttattgactgtgtctggcagatgacaagacagtttcctaccgcatttgaattcaatgagtattttctcattaccattttggaccacctatacagctgcttattcggaacattcctctgtaatagtgaacaacagagaggaaaagagaatcttcctaaaaggactgtgtcactgtggtcttacataaacagccagctggaagacttcactaatcctctctatgggagctattccaatcatgtcctttatccagtagccagcatgcgccacctagagctctgggtgggatattacataaggtggaatccacggatgaaaccacaggaacctattcacaacagatacaaagaacttcttgctaaacgagcagagcttcagaaaaaagtagaggaactacagagagagatttctaaccgatcaacctcatcctcagagagagccagctctcctgcacagtgtgtcactcctgtccaaactgttgtataaaggactgtaagatcaggggcatcattgctatacactcttgattacactggcagctctatgagtagaaagtcttcggaatttagaacccatctatgagagaaagttcagtcactttatttattttaaatctctctaggatgagtttagaactgtagcagtgcaggtggcttaagtgaagtaactccatatgtaattacatgattatgatactaatcttttaagtatccaaagaatattaaaatacttcaatcctggattcacagtgggaacaagtttctattaaaaggcaaatgctgttacaaatttttggcatctggtaatattaaaaccattttagaaatacactctgtgctcactgtgcagaggaacatcagttttcaaaccaacactgaaattctgtggcatcacatatattgggccttgatgtcatgacagatcaaaatcatttgatatccctttctccattctaggtttttctttttttcagtaactgatttaccttgatcacttttcaacttccatattcttcatatagtaaaaggcaaagtgttgaagatactacggtgtggtagtagttgaaaattattgccgtcattatttacatacttaagacatattagcaagttgatccaaaatgggaggccttatagatgtgcttgggggaaaatgaaggggagaaagtagccatacaggagttcaaagaattccatgcccttcagattagcccaattaccagaaacatcatgaaagatattttaaaaactaattatttactacagtgtatttcacttgtcttgtgtgtctgaacacacagaagctaattagcaagtttttaagaagtatttaaaaatcttactaggattgacattttttctgaattctgtataaatagcttatagtgagaagtactgtgctcaaattttacatttttttcctttgcaaattctgtaatttcactcaacgattaagtctaccaaagaacacactgcatgtaaaagatgtattacaatctcaaagccagtaaaagaaatcttgcttcactgttcacctgctacaagtaagagtttggtgctggtagaaacatttgactctgatgtctattttattctacataagagccatatgtaatgtactgtaacaaaggagcttcttgtccccttggtcttttaattaaaagaaattccaactgacttttaaactttgttcttgtccaaagttgccatttcttttttttccccagaaatatttggaaattattggaggaatatgcaccccagatgaaaatgttcagtttgtacccatttttccttaaccaacacccaaatcaaacaattaaaatatacagtgtttttccactcactaattcactatacagagagtctgaaccttagcctccctcttggtcttgcagtgaggaagtttctattagtatatccaatttagcaaaattggtaccaaaatgatttctttggtaattgtgtgaaatataagctttttaacagggcatttaagtggctagcaaatcagtaattaaaaattaagctttctactccaagtatttcacaaacgcatctgccattttcctcatttaaaccttggttatcttggcctgataccacataaaagaatgtagaatggctgaagagatcaagaatttaaagcttctagtcttaacatacttgcatccacttcaaattcaaatcaaaagccagggaaatctaagtgcaaccctaccacttctctgctgagaaccttccagtggttcccctcaccttctgcagaagtctccaatatggagtacatgcacttgggcatttaatatataccactggtgtgtgtgggagggagggaggaggaatactagccctttttatatatttacacaagcaaaacttttaaatatttgaattgacagttacatgtttcataactttgtatgtctattggttgtgcaggtgtaattttttccctttttgattagggttacaaaatttagagaccagtatgattaagttgaagctccttagcctccttcgacctagtctctgcatacctcaacttttacgtaccaatgctactctgctgttcacaattgcctcatgtaatctgcagattcctgcctccccactttggttcagtctgtcttgtgcacctggaacaactgttctcccttgtgactaattcctattttctagagtttaggcatcatctcttcctttgggaagttatctgattcacgactgccttctctgacatccccaccttcctctgtgcccccatagcactgtgtataccgctactaccactgcaattcacattatattggaatgaacaattcacatgtctaccacaagtctgtaaacataaccttatttgaaatgaattgcaataaagctctgttacaacgtaa

SEQ ID NO: 6 - DNA, 22 bp, Artificial Sequence
  forward primer 5'UTR MTMR2
agcggcctccagtttctcgcgc

SEQ ID NO: 7 - DNA, 26 bp, artificial
  reverse primer exon 3
tctctcctggaagcagggctggttcc

SEQ ID NO: 8 - DNA, 20 bp, Artificial Sequence
  forward primer mouse MTMR2 V1
gactcactgtccagtgcttc

SEQ ID NO: 9 - DNA, 18 bp, Artificial Sequence
  reverse primer mouse MTMR2 V1
cctccctcaggaccctca

SEQ ID NO: 10 - DNA, 20 bp, Artificial Sequence
  forward primer mouse MTMR2 V2
gactcactgtccagtgcttc

SEQ ID NO: 11 - DNA, 18 bp, Artificial Sequence
  reverse primer mouse MTMR2 V2
cagctgggcactccctca

SEQ ID NO: 12 - DNA, 33 bp, Artificial Sequence
  forward primer mouse MTMR2 V3
aagataaaacatctcaaaaattataattgcttc

SEQ ID NO: 13 - DNA, 18 bp, Artificial Sequence
  reverse primer mouse MTMR2 V3
cagctgggcactccctca

SEQ ID NO: 14 - DNA, 33 bp, Artificial Sequence; identical to SEQ ID NO: 12
  forward primer mouse MTMR2 V4

SEQ ID NO: 15 - DNA, 20 bp, Artificial Sequence
  reverse primer mouse MTMR2 V4
gactcactgtccagtgcttc

SEQ ID NO: 16 - DNA, 20 bp, Artificial Sequence
  forward primer total mouse MTMR2
tcctgtgtctaatggcttgc

SEQ ID NO: 17 - DNA, 20 bp, Artificial Sequence
  reverse primer total mouse MTMR2
aaccaagagggcaggatatg

SEQ ID NO: 18 - DNA, 19 bp, Artificial Sequence
  forward primer human MTMR2 V1
actccttgtccagtgcctc

SEQ ID NO: 19 - DNA, 18 bp, Artificial Sequence
  reverse primer human MTMR2 V1
gactccctcaggaccctc

SEQ ID NO: 20 - DNA, 33 bp, Artificial Sequence
  forward primer human MTMR2 V2
aagataaaacatctcaaaaattataattgcctc

SEQ ID NO: 21 - DNA, 18 bp, Artificial Sequence
  reverse primer human MTMR2 V2
gactccctcaggaccctc

SEQ ID NO: 22 - DNA, 33 bp, Artificial Sequence; identical to SEQ ID NO: 20
  forward primer human MTMR2 V3

SEQ ID NO: 23 - DNA, 18 bp, Artificial Sequence
  reverse primer human MTMR2 V3
gagcgagactccctcctc

SEQ ID NO: 24 - DNA, 33 bp, Artificial Sequence; identical to SEQ ID NO: 20
  forward primer human MTMR2 V4

SEQ ID NO: 25 - DNA, 18 bp, Artificial Sequence
  reverse primer human MTMR2 V4
ctggactgcatgggcctc

SEQ ID NO: 26 - DNA, 23 bp, Artificial Sequence
  forward primer total human MTMR2
tttcctgtctctaataacctgcc

SEQ ID NO: 27 - DNA, 18 bp, Artificial Sequence
  reverse primer total human MTMR2
ccaggagggcagggtatg

SEQ ID NO: 28 - DNA, 71 bp, Homo sapiens
ttaatgtgttaagaaccattgacatttgaagatcatcagaagtgaagataaaacatctcaaaaattataat

SEQ ID NO: 29 - DNA, 105 bp, Homo sapiens
gagtgcccagctgcttgggttttagttgatgccagacatagtcaagttgacagccaagattagccatcacaccagtgttctatcctgttgaatccaattctatag